European Patent Application EP 4 350 005 A1, published April 10, 2024. Title: Method for screening externally introduced mRNA that can exist for a long time in a cell. Applicant: RNAGENE Inc. The sequence listing filed with the application follows.

SEQUENCE LISTING (40 sequences)

SEQ ID NO: 1 - DNA, 760 bp, Artificial Sequence
  WT_Template
agatctaatacgactcactatagggaaataagagagaaaagaagagtaagaagaaatataagagaattcgccaccatgggagtgaaagttctttttgcccttatttgtattgctgtggccgaggccaaaccaactgaaaacaatgaagatttcaacattgtagctgtagctagcaactttgctacaacggatctcgatgctgaccgtggtaaattgcccggaaaaaaattaccacttgaggtactcaaagaaatggaagccaatgctaggaaagctggctgcactaggggatgtctgatatgcctgtcacacatcaagtgtacacccaaaatgaagaagtttatcccaggaagatgccacacctatgaaggagacaaagaaagtgcacagggaggaataggagaggctattgttgacattcctgaaattcctgggtttaaggatttggaacccatggaacaattcattgcacaagttgacctatgtgtagactgcacaactggatgcctcaaaggtcttgccaatgtgcaatgttctgatttactcaagaaatggctgccacaaagatgtgcaacttttgctagcaaaattcaaggccaagtggacaaaataaagggtgccggtggtgattaaggatccgctgccttctgcggggcttgccttctggccatgcccttcttctctcccttgcacctgtacctcttggtctttgaataaagcctgagtaggaagaatattaaaaaaaaaaaaaaaaaagctt

SEQ ID NO: 2 - DNA, 760 bp, Artificial Sequence
  variation_Template
agatctaatacgactcactatagggaaataagagagaaaagaagagtaagaagaaatataagagaattcgccaccatgggngtnaargtnctnttygcnctnathtgyathgcngtngcngargcnaarccnacngaraayaaygargayttyaayathgtngcngtngcntcnaactttgctacaacggatctngaygcngaycgnggnaarctnccnggnaaraarctnccnctngargtnctnaargaratggargcnaaygcncgnaargcnggntgyacncgnggntgtctgatatgcctgtcacayathaartgyacnccnaaratgaaraarttyathccnggncgntgycayacntaygarggngayaargartcngcncarggnggnathggngargcnattgttgacattcctgaaathccnggnttyaargayctngarccnatggarcarttyathgcncargtngayctntgygtngaytgyacnacnggntgyctnaarggnctngcnaaygtgcaatgttctgatttactnaaraartggctnccncarcgntgygcnacnttygcntcnaarathcarggncargtngayaarathaarggngcnggnggngaytaaggatccgctgccttctgcggggcttgccttctggccatgcccttcttctctcccttgcacctgtacctcttggtctttgaataaagcctgagtaggaagaatattaaaaaaaaaaaaaaaaaagctt

SEQ ID NO: 3 - DNA, 75 bp, Artificial Sequence
  PM_Rpic_GL_F1
agatctaatacgactcactatagggaaataagagagaaaagaagagtaagaagaaatataagagaattcgccacc

SEQ ID NO: 4 - DNA, 135 bp, Artificial Sequence
  PM_Rpic_GL_R1
atccgttgtagcaaagttngangcnacngcnacdatrttraartcytcrttrttytcngtnggyttngcytcngcnacngcdatrcadatnagngcraanagnacyttnacncccatggtggcgaattctcttat

SEQ ID NO: 5 - DNA, 135 bp, Artificial Sequence
  PM_Rpic_GL_R2
tgacaggcatatcagacanccncgngtrcanccngcyttncgngcrttngcytccatytcyttnagnacytcnagnggnagyttyttnccnggnagyttnccncgrtcngcrtcnagatccgttgtagcaaagtt

SEQ ID NO: 6 - DNA, 135 bp, Artificial Sequence
  PM_Rpic_GL_R3
ttcaggaatgtcaacaatngcytcnccdatnccnccytgngcngaytcyttrtcnccytcrtangtrtgrcancgnccnggdatraayttyttcatyttnggngtrcayttdatrtgtgacaggcatatcagaca

SEQ ID NO: 7 - DNA, 135 bp, Artificial Sequence
  PM_Rpic_GL_R4
taaatcagaacattgcacrttngcnagnccyttnagrcanccngtngtrcartcnacrcanagrtcnacytgngcdatraaytgytccatnggytcnagrtcyttraanccnggdatttcaggaatgtcaacaat

SEQ ID NO: 8 - DNA, 126 bp, Artificial Sequence
  PM_Rpic_GL_R5
gcagaaggcagcggatccttartcnccnccngcnccyttdatyttrtcnacytgnccytgdatyttngangcraangtngcrcancgytgnggnagccayttyttnagtaaatcagaacattgcac

SEQ ID NO: 9 - DNA, 92 bp, Artificial Sequence
  PM_Rpic_GL_R6
ctcaggctttattcaaagaccaagaggtacaggtgcaagggagagaagaagggcatggccagaaggcaagccccgcagaaggcagcggatcc

SEQ ID NO: 10 - DNA, 99 bp, Artificial Sequence
  seq32
tttttttttttttttttttttttttttttttttttttttttttttttttttttttttttttttttaatattcttcctactcaggctttattcaaagacc

SEQ ID NO: 11 - DNA, 33 bp, Artificial Sequence
  seq30
agatctaatacgactcactatagggaaataaga

SEQ ID NO: 12 - DNA, 192 bp, Artificial Sequence
  PCR_product_1
agatctaatacgactcactatagggaaataagagagaaaagaagagtaagaagaaatataagagaattcgccaccatgggngtnaargtnctnttygcnctnathtgyathgcngtngcngargcnaarccnacngaraayaaygargayttyaayathgtngcngtngcntcnaactttgctacaacggat

SEQ ID NO: 13 - DNA, 309 bp, Artificial Sequence
  PCR_product_2
agatctaatacgactcactatagggaaataagagagaaaagaagagtaagaagaaatataagagaattcgccaccatgggngtnaargtnctnttygcnctnathtgyathgcngtngcngargcnaarccnacngaraayaaygargayttyaayathgtngcngtngcntcnaactttgctacaacggatctngaygcngaycgnggnaarctnccnggnaaraarctnccnctngargtnctnaargaratggargcnaaygcncgnaargcnggntgyacncgnggntgtctgatatgcctgtca

SEQ ID NO: 14 - DNA, 426 bp, Artificial Sequence
  PCR_product_3
agatctaatacgactcactatagggaaataagagagaaaagaagagtaagaagaaatataagagaattcgccaccatgggngtnaargtnctnttygcnctnathtgyathgcngtngcngargcnaarccnacngaraayaaygargayttyaayathgtngcngtngcntcnaactttgctacaacggatctngaygcngaycgnggnaarctnccnggnaaraarctnccnctngargtnctnaargaratggargcnaaygcncgnaargcnggntgyacncgnggntgtctgatatgcctgtcacayathaartgyacnccnaaratgaaraarttyathccnggncgntgycayacntaygarggngayaargartcngcncarggnggnathggngargcnattgttgacattcctgaa

SEQ ID NO: 15 - DNA, 543 bp, Artificial Sequence
  PCR_product_4
agatctaatacgactcactatagggaaataagagagaaaagaagagtaagaagaaatataagagaattcgccaccatgggngtnaargtnctnttygcnctnathtgyathgcngtngcngargcnaarccnacngaraayaaygargayttyaayathgtngcngtngcntcnaactttgctacaacggatctngaygcngaycgnggnaarctnccnggnaaraarctnccnctngargtnctnaargaratggargcnaaygcncgnaargcnggntgyacncgnggntgtctgatatgcctgtcacayathaartgyacnccnaaratgaaraarttyathccnggncgntgycayacntaygarggngayaargartcngcncarggnggnathggngargcnattgttgacattcctgaaathccnggnttyaargayctngarccnatggarcarttyathgcncargtngayctntgygtngaytgyacnacnggntgyctnaarggnctngcnaaygtgcaatgttctgattta

SEQ ID NO: 16 - DNA, 651 bp, Artificial Sequence
  PCR_product_5
agatctaatacgactcactatagggaaataagagagaaaagaagagtaagaagaaatataagagaattcgccaccatgggngtnaargtnctnttygcnctnathtgyathgcngtngcngargcnaarccnacngaraayaaygargayttyaayathgtngcngtngcntcnaactttgctacaacggatctngaygcngaycgnggnaarctnccnggnaaraarctnccnctngargtnctnaargaratggargcnaaygcncgnaargcnggntgyacncgnggntgtctgatatgcctgtcacayathaartgyacnccnaaratgaaraarttyathccnggncgntgycayacntaygarggngayaargartcngcncarggnggnathggngargcnattgttgacattcctgaaathccnggnttyaargayctngarccnatggarcarttyathgcncargtngayctntgygtngaytgyacnacnggntgyctnaarggnctngcnaaygtgcaatgttctgatttactnaaraartggctnccncarcgntgygcnacnttygcntcnaarathcarggncargtngayaarathaarggngcnggnggngaytaaggatccgctgccttctgc

SEQ ID NO: 17 - DNA, 725 bp, Artificial Sequence
  PCR_product_6
agatctaatacgactcactatagggaaataagagagaaaagaagagtaagaagaaatataagagaattcgccaccatgggngtnaargtnctnttygcnctnathtgyathgcngtngcngargcnaarccnacngaraayaaygargayttyaayathgtngcngtngcntcnaactttgctacaacggatctngaygcngaycgnggnaarctnccnggnaaraarctnccnctngargtnctnaargaratggargcnaaygcncgnaargcnggntgyacncgnggntgtctgatatgcctgtcacayathaartgyacnccnaaratgaaraarttyathccnggncgntgycayacntaygarggngayaargartcngcncarggnggnathggngargcnattgttgacattcctgaaathccnggnttyaargayctngarccnatggarcarttyathgcncargtngayctntgygtngaytgyacnacnggntgyctnaarggnctngcnaaygtgcaatgttctgatttactnaaraartggctnccncarcgntgygcnacnttygcntcnaarathcarggncargtngayaarathaarggngcnggnggngaytaaggatccgctgccttctgcggggcttgccttctggccatgcccttcttctctcccttgcacctgtacctcttggtctttgaataaagcctgag

SEQ ID NO: 18 - DNA, 803 bp, Artificial Sequence
  PCR_product_7
agatctaatacgactcactatagggaaataagagagaaaagaagagtaagaagaaatataagagaattcgccaccatgggngtnaargtnctnttygcnctnathtgyathgcngtngcngargcnaarccnacngaraayaaygargayttyaayathgtngcngtngcntcnaactttgctacaacggatctngaygcngaycgnggnaarctnccnggnaaraarctnccnctngargtnctnaargaratggargcnaaygcncgnaargcnggntgyacncgnggntgtctgatatgcctgtcacayathaartgyacnccnaaratgaaraarttyathccnggncgntgycayacntaygarggngayaargartcngcncarggnggnathggngargcnattgttgacattcctgaaathccnggnttyaargayctngarccnatggarcarttyathgcncargtngayctntgygtngaytgyacnacnggntgyctnaarggnctngcnaaygtgcaatgttctgatttactnaaraartggctnccncarcgntgygcnacnttygcntcnaarathcarggncargtngayaarathaarggngcnggnggngaytaaggatccgctgccttctgcggggcttgccttctggccatgcccttcttctctcccttgcacctgtacctcttggtctttgaataaagcctgagtaggaagaatattaaaaaaaaaaaaaaaaaaaaaaaaaaaaaaaaaaaaaaaaaaaaaaaaaaaaaaaaaaaaaaaaa

SEQ ID NO: 19 - DNA, 558 bp, Artificial Sequence
  RPIC_GL_3
atgggcgtcaaagtactcttcgccctcatttgtattgcggtcgcggaggcgaagccaacagagaataacgaggactttaacatagtagcggtggcatcgaactttgctacaacggatctcgacgccgatcgaggaaaactccccggaaaaaaactaccgctagaggtactaaaggaaatggaagcaaacgctcgtaaagccggctgtacacgtggctgtctgatatgcctgtcacacatcaaatgcacgcctaaaatgaagaagttcataccaggccgctgccacacgtacgagggagataaagagtcggcacagggaggcattggggaggccattgttgacattcctgaaataccggggttcaaggatcttgaacccatggagcaattcatcgcgcaagtcgacctgtgcgtggactgcaccactggatgcctgaagggtctcgctaatgtgcaatgttctgatttactaaagaaatggctcccacaacgatgtgcgacgttcgcttcaaagattcagggccaagtagataaaatcaaaggagcaggaggagactaa

SEQ ID NO: 20 - DNA, 558 bp, Artificial Sequence
  RPIC_GL_5
atgggagtgaaagtgctcttcgcacttatatgcatcgcggttgccgaagctaaaccaacggaaaataatgaagactttaacattgtagccgtagcgtccaactttgctacaacggatctcgatgctgatcgaggcaaactgcccggtaaaaaactcccccttgaggtgctcaaagaaatggaagccaacgctcggaaagccggctgcacacgggggtgtctgatatgcctgtcacacatcaaatgcactcccaaaatgaaaaaattcatccctggtcgatgccacacatacgaaggcgacaaggaatcagcgcagggaggcataggcgaggcgattgttgacattcctgaaatacccggcttcaaggacctcgagcccatggaacagttcatagcccaagtcgatctctgcgtcgactgcacaaccggttgcctcaaaggactagcgaacgtgcaatgttctgatttacttaagaaatggctacctcaacgttgcgctaccttcgcgtcaaagatacaaggtcaggtcgataagataaaaggcgccggtggcgattaa

SEQ ID NO: 21 - DNA, 558 bp, Artificial Sequence
  RPIC_GL_7
atgggagtgaaagtgcttttcgcacttatatgcatcgcggttgccgaagctaaaccaacggaaaataatgaagactttaacattgtagccgtagcgtccaactttgctacaacggatctcgatgctgatcgaggcaaactgcccggtaaaaaactcccccttgaggtgctcaaagaaatggaagccaacgctcggaaagccggctgcacacgggggtgtctgatatgcctgtcacacatcaaatgcactcccaaaatgaaaaaattcatccctggtcgatgccacacatacgaaggcgacaaggaatcagcgcagggaggcataggcgaggcgattgttgacattcctgaaatacccggcttcaaggacctcgagcccatggaacagttcatagcccaagtcgatctctgcgtcgactgcacaaccggttgcctcaaaggactagcgaacgtgcaatgttctgatttacttaagaaatggctacctcaacgttgcgctaccttcgcgtcaaagatacaaggtcaggtcgataagataaaaggcgccggtggcgattaa

SEQ ID NO: 22 - DNA, 558 bp, Artificial Sequence
  RPIC_GL_9
atgggagtgaaagtgctcttcgcacttatatgcatcgcggttgccgaagctaaaccaacggaaaataatgaagactttaacattgtagccgtagcgtccaactttgctacaacggatctcgatgctgatcgaggcaaactgcccggtaaaaaactcccccttgaggtgctcaaagaaatggaagccaacgctaggaaagccggctgcacacgggggtgtctgatatgcctgtcacacatcaaatgcactcccaaaatgaaaaaattcatccctggtcgatgccacacatacgaaggcgacaaggaatcagcgcagggaggcataggcgaggcgattgttgacattcctgaaatacccggcttcaaggacctcgagcccatggaacagttcatagcccaagtcgatctctgcgtcgactgcacaaccggttgcctcaaaggactagcgaacgtgcaatgttctgatttacttaagaaatggctacctcaacgttgcgctaccttcgcgtcaaagatacaaggtcaggtcgataagataaaaggcgccggtggcgattaa

SEQ ID NO: 23 - DNA, 558 bp, Artificial Sequence
  RPIC_GL_15
atgggcgtaaaagtgctcttcgcgcttatttgcatcgctgtcgctgaggccaaaccgacagaaaacaatgaggatttcaacatagtcgcggtagcatcaaactttgctacaacggatctcgacgccgaccgaggcaagctgcctgggaagaagctcccgcttgaagtgctaaaagagatggaagcgaacgcccgaaaagcgggatgtacccgtggatgtctgatatgcctgtcacacatcaagtgcacacccaagatgaagaagttcatccctggacggtgccacacctacgaaggagacaaagaatcggcccaaggcggaataggagaggcaattgttgacattcctgaaatcccaggatttaaggacctagaacccatggaacagttcatcgcacaggtggacctatgtgtggattgcacaaccggatgcctcaaaggtctggcgaatgtgcaatgttctgatttactgaaaaaatggctcccccagcgctgtgccactttcgcctcaaagattcagggccaagtcgacaaaatcaagggtgcaggtggcgactaa

SEQ ID NO: 24 - DNA, 558 bp, Artificial Sequence; identical to SEQ ID NO: 22
  RPIC_GL_28

SEQ ID NO: 25 - DNA, 558 bp, Artificial Sequence
  RPIC_GL_32
atgggcgtgaaagtgctgtttgctctgatctgtatagcagtagctgaggccaagccaaccgagaacaacgaggatttcaacatagttgctgtcgcctccaactttgctacaacggatcttgacgctgaccgaggtaaactaccaggcaagaagctccccctcgaagtgctaaaggagatggaagcaaacgcacgcaaggcgggttgcacacggggttgtctgatatgcctgtcacacatcaaatgcacgcccaagatgaaaaaatttattcccggccgatgccacacatacgaaggcgataaagagtccgcacaaggcggtataggggaagctattgttgacattcctgaaattcccggattcaaagatctcgagcctatggagcagttcatcgcacaggtcgacctgtgcgtagactgtactacaggctgtctaaaaggactagccaacgtgcaatgttctgatttactcaagaagtggcttccccagcgatgcgcgacattcgcatcaaagattcaagggcaagtcgacaaaataaagggagccggaggagactaa

SEQ ID NO: 26 - DNA, 558 bp, Artificial Sequence; identical to SEQ ID NO: 19
  RPIC_GL_34

SEQ ID NO: 27 - DNA, 887 bp, Artificial Sequence
  C19_WT
agatcttaatacgactcactatagggaaataagacgcgcctagcagtgtcccagccgggttcgtgtcgccgaattcgccaccatgggagtgaaagttctttttgcccttatttgtattgctgtggccgaggccggcgccgccccgacggaatccatagtgcgctttcccaacattacaaacctctgtccttttggggaagtatttaacgcaacgagattcgccagtgtttatgcgtggaaccgcaaaagaatatccaactgtgttgccgactatagtgttctgtataactctgcctcctttagcactttcaagtgttacggagtaagtcctacaaagttgaatgatttgtgctttacaaatgtgtacgcagattcattcgtcatcaggggggacgaggttcgacagatagcaccgggtcaaactggcaaaatagcggattacaattacaagttgccggatgattttacgggttgtgtcatagcgtggaactccaacaatttggattcaaaagtaggaggtaactataactacctttatcgactttttcgcaagagcaaccttaaaccttttgagagagatataagtacagagatttaccaagccggaagtactccttgcaacggagtggaaggattcaattgttacttcccattgcagtcctacggctttcagccaactaatggcgttggatatcagccttatcgcgtcgtagtgttgagtttcgagttgttgcacgcccctgcgactgtggccctggttccaaggggctcttcagctcatcatcaccatcatcatcatcaccatcactgaggatcccctcgccccggacctgccctcccgccaggtgcacccacctgcaataaatgcagcgaagccgggaaatatt

SEQ ID NO: 28 - DNA, 887 bp, Artificial Sequence
  C19_#15
agatcttaatacgactcactatagggaaataagacgcgcctagcagtgtcccagccgggttcgtgtcgccgaattcgccaccatgggggttaaggtgcttttcgccctcatttgcatcgctgtggcagaggcaggcgccgccccgacggaatccatagtgcgattcccaaatataacaaacctctgcccgtttggcgaagtgttcaacgcaacgagattcgccagtgtgtatgcatggaaccggaaacgtatttcgaattgcgtcgccgactatagtgttctgtataactctgcctctttctctacgtttaaatgttacggcgtttcaccgaccaagctaaacgatttgtgctttacaaatgtgtatgcggattcttttgtaattcggggcgatgaggttcgccaaatagctccgggtcaaactggcaaaatagctgactacaactacaagcttcctgacgattttaccgggtgtgttatcgcgtggaactccaacaatttggactcaaaagttggcgggaactacaactacctttaccggctttttcgaaagagcaaccttaaaccttttgaacgcgatatatcgacggagatctatcaggctggatccacgccatgcaacggagtggaaggattcaattgctatttcccgctccaatcctacggcttccagccaacaaacggagtgggatatcagccttatcgcgtcgttgtactttcgtttgagctactacacgcgccggcaactatggccctggttccaaggggctcttcagctcatcatcaccatcatcatcatcaccatcactgaggatcccctcgccccggacctgccctcccgccaggtgcacccacctgcaataaatgcagcgaagccgggaaatatt

SEQ ID NO: 29 - DNA, 887 bp, Artificial Sequence
  C19_#27
agatcttaatacgactcactatagggaaataagacgcgcctagcagtgtcccagccgggttcgtgtcgccgaattcgccaccatgggcgtcaaggtcctattcgcgctgatatgcatcgctgtggcagaagcaggcgccgccccgacggaatccatagttcgcttccctaatataaccaacctctgcccatttggtgaggtgttcaacgcaacgagattcgccagtgtgtacgcatggaatcggaagcggatttctaactgcgtggcagactacagtgttctgtataactctgcctcgttctctactttcaagtgctacggtgtgtcacctaccaagcttaatgatttgtgctttacaaatgtgtacgctgattcatttgtcattcggggagatgaggttcgacaaatcgcaccgggtcaaactggcaaaatagctgattataactataagctgccggatgattttactgggtgtgtcattgcgtggaactccaacaatttggattctaaagtgggcggcaactacaactatctgtatcgcctatttcggaagagcaaccttaaaccttttgaacgggacatatcaaccgaaatataccaagcaggctccaccccttgtaacggagtggaaggattcaattgttacttcccccttcagtcatatgggtttcagccaactaacggagtcggatatcagccttatcgcgtcgtggtactttcttttgaactcctgcatgcgccagctaccgttgcactggttccaaggggctcttcagctcatcatcaccatcatcatcatcaccatcactgaggatcccctcgccccggacctgccctcccgccaggtgcacccacctgcaataaatgcagcgaagccgggaaatatt

SEQ ID NO: 30 - DNA, 887 bp, Artificial Sequence
  C19_#57
agatcttaatacgactcactatagggaaataagacgcgcctagcagtgtcccagccgggttcgtgtcgccgaattcgccaccatgggagtgaaagtacttttcgccctgatttgtatagccgtggctgaagcaggcgccgccccgacggaatccatagtacgattcccaaacattactaatctttgcccattcggtgaagtctttaacgcaacgagattcgccagtgtttacgcgtggaaccgtaagcgaatctccaattgcgttgctgactatagtgttctgtataactctgcctcattctcgactttcaagtgttatggcgtctcgcctactaagctgaatgatttgtgctttacaaatgtgtatgccgattcgttcgtcatccgcggtgacgaagtgcgtcaaatcgctccgggtcaaactggcaaaatagcggactataactataagctaccggacgattttacggggtgcgtcatcgcgtggaactccaacaatttggactctaaggtcggcggcaattacaactatctctaccgacttttccgcaagagcaaccttaaaccttttgaacgagatatctcaacggagatttatcaggctggttctacaccgtgcaacggagtggaaggattcaattgctattttccgctccaatcttacggtttccaaccgactaacggggtgggatatcagccttatcgcgtcgtagtcctttccttcgaactcctccatgcgccagcgactgtcgctctggttccaaggggctcttcagctcatcatcaccatcatcatcatcaccatcactgaggatcccctcgccccggacctgccctcccgccaggtgcacccacctgcaataaatgcagcgaagccgggaaatatt

SEQ ID NO: 31 - DNA, 887 bp, Artificial Sequence
  C19_#79
agatcttaatccgactcactatagggaaataagacgcgcctagcagtgtcccagccgggttcgtgtcgccgaattcgccaccatgggtgtgaaagtactcttcgccctcatctgcattgcggtagctgaggcgggcgccgccccgacggaatccatagtgcggttccccaatattaccaacctttgtccgtttggagaggtcttcaacgcaacgagattcgccagtgtatacgcatggaaccgcaaacggatatccaactgcgtcgctgattacagtgttctgtataactctgcctctttttccacctttaagtgctatggggtatctcctacgaagctcaatgatttgtgctttacaaatgtgtacgcggactcctttgtcattcgtggtgatgaagtccgacaaatcgcaccgggtcaaactggcaaaatagcggactataattacaagcttcccgacgattttacaggctgcgtcattgcgtggaactccaacaatttggattccaaagtcggtggtaattacaattacctgtatcgtctctttcgaaagagcaaccttaaaccttttgagcgggatatatcaacggagatttaccaagccggatccaccccttgtaacggagtggaaggattcaattgctacttcccccttcaatcatatggattccagcccactaatggcgtcggatatcagccttatcgcgtcgttgtcctttcttttgaactgctgcatgcacctgcgaccgtcgcgctggttccaaggggctcttcagctcatcatcaccatcatcatcatcaccatcactgaggatcccctcgccccggacctgccctcccgccaggtgcacccacctgcaataaatgcagcgaagccgggaaatatt

SEQ ID NO: 32 - DNA, 887 bp, Artificial Sequence
  C19_#80
agatcttaatacgactcactatagggaaataagacgcgcctagcagtgtcccagccgggttcgtgtcgccgaattcgccaccatgggagtaaaagtactgtttgccctaatctgcatcgccgttgcggaggcaggcgccgccccgacggaatccatagtgcgattccccaacattaccaatctgtgcccttttggtgaggtgtttaacgcaacgagattcgccagtgtatatgcttggaatcgcaagcgaatctcaaactgtgtggccgactacagtgttctgtataactctgcctcgttttctacgtttaagtgctacggtgtgtctcctactaagctcaacgatttgtgctttacaaatgtgtacgccgattcattcgtaatacgaggtgacgaagttcgccaaatcgcgccgggtcaaactggcaaaatagcggactataactacaagcttcctgatgatttcaccggttgtgtgatagcgtggaactccaacaatttggattccaaagtaggcggaaactataactatctataccgcctattccgaaagagcaaccttaaaccttttgaacgggatatttcgactgagatctatcaggcaggttcgactccatgtaacggagtggaaggattcaattgctacttccccctgcaatcatatggatttcaaccaactaacggagttggatatcagccttatcgcgtcgtggtcctgtcgttcgaacttcttcatgctccagctactgtcgctctggttccaaggggctcttcagctcatcatcaccatcatcatcatcaccatcactgaggatcccctcgccccggacctgccctcccgccaggtgcacccacctgcaataaatgcagcgaagccgggaaatatt

SEQ ID NO: 33 - DNA, 887 bp, Artificial Sequence
  C19_#93
agatcttaatacgactcactatagggaaataagacgcgcctagcagtgtcccagccgggttcgtgtcgccgaattcgccaccatgggggttaaagtactcttcgcgctcatatgtattgcggtagccgaggcaggcgccgccccgacggaatccatagttcgtttccccaacataacgaatctctgtccatttggagaggtctttaacgcaacgagattcgccagtgtttacgcctggaatcgcaaacggatttcaaactgcgttgccgattacagtgttctgtataactctgcctctttctctacgttcaagtgttatggggtatcgccaaccaagctaaatgatttgtgctttacaaatgtgtacgcggactcattcgtgatccgaggtgacgaggtccgacaaatagcaccgggtcaaactggcaaaatagccgattataattacaagctgcctgatgatttcacgggatgtgtaatagcgtggaactccaacaatttggattctaaagtcggcggcaactataattatctgtatcggctattccgaaagagcaaccttaaaccttttgagcgggatatttctactgaaatatatcaggcagggtcgacgccttgtaacggagtggaaggattcaattgttactttcctctacaatcctacggcttccaaccgactaatggcgtgggatatcagccttatcgcgtcgttgtactctctttcgagctgctccatgctcccgctacagttgcgctggttccaaggggctcttcagctcatcatcaccatcatcatcatcaccatcactgaggatcccctcgccccggacctgccctcccgccaggtgcacccacctgcaataaatgcagcgaagccgggaaatatt

SEQ ID NO: 34 - DNA, 887 bp, Artificial Sequence
  C19_#114
agatcttaatacgactcactatagggaaataagacgcgcctagcagtgtcccagccgggttcgtgtcgccgaattcgccaccatgggtgtcaaagtcctgttcgctctaatctgtattgccgtagcggaggcaggcgccgccccgacggaatccatagtgcggtttcccaatatcacgaacctctgtccatttggtgaagtatttaacgcaacgagattcgccagtgtctacgcatggaatcgaaaacgtatctccaactgtgtagccgactatagtgttctgtataactctgcctcgttctcgacttttaagtgttatggggtttcgccgacgaagcttaatgatttgtgctttacaaatgtgtatgcggactcgttcgtaattcgaggcgacgaagtgcgccagatagcgccgggtcaaactggcaaaatagctgactacaactataagcttccggatgatttcactggttgtgtgatagcgtggaactccaacaatttggactctaaggtcggcggtaattacaactacctctatcgcctatttcgaaagagcaaccttaaaccttttgagcgtgatatatctactgaaatttaccaggctggatctacgccgtgtaacggagtggaaggattcaattgttactttcctctccagtcttacggtttccaaccgacaaacggcgtgggatatcagccttatcgcgtcgttgtactgtcgttcgagctgctgcacgctccggccactgtagcgctggttccaaggggctcttcagctcatcatcaccatcatcatcatcaccatcactgaggatcccctcgccccggacctgccctcccgccaggtgcacccacctgcaataaatgcagcgaagccgggaaatatt

SEQ ID NO: 35 - DNA, 1703 bp, Artificial Sequence
  C19DP-MR-#6
agatcttaatacgactcactatagggaaataagacgcgcctagcagtgtcccagccgggttcgtgtcgccgaattcgccaccatgggtgtaaaggttctgtttgcactcatctgcatcgccgtcgcagaagcaggcgccgccccgacggagtcgatcgtccgattcccaaacataacaaacctatgtccatttggagaggtttttaacgcgacacgttttgcgtcggtttatgcgtggaatcgcaaaagaatatccaactgtgtcgccgattattccgtactatataattccgcttcattctcaacattcaaatgctatggcgtatcacccacgaaactaaatgatctttgcttcacaaatgtatatgctgattcattcgtcattcgcggagacgaagtacgtcaaatcgcgcccggacaaactggcaacatagcggattacaattacaagctcccagacgactttacagggtgtgtcattgcttggaattccaacaatctagactcaaaagtaggagggaactataactatcggtatcgtctgtttcggaaatctaacctaaaaccgtttgaacgagacatatcaactgaaatttaccaagccggaagtaagccttgcaacggtgtcgagggtttcaattgttattttccccttcaatcatatggatttcaacctacaaacggagtcggatatcaaccataccgagttgtagtcctctcctttgaacttcttcatgcacctgcaacggttacctcagctgaggcagcggccaaagaggctgcagctaaagaagcagcagcaaaggaagccgcggctaaagctctagaagctgaagctgcagcgaaagaagcagcagctaaagaagctgccgcaaaagaagcagctgctaaagcagaagctaagccgtccgggtccgtcgtggaacaagctgaaggagtcgaatgcgatttctctccgcttctgtcaggcaccccaccacaggtatataacttcaaacgactcgtgttcactaattgtaattataatctaacaaagcttctttcactcttttcagtcaatgatttcacctgctctcaaatatcgccagctgctatagcatcaaattgttattcttctctaatcctagattacttcagctatccgttgtccatgaaatcagatctatcggtctcctctgccggccctatctcacaatttaattacaaacagtctttctcaaatcctacctgtctaattctcgcaaccgttccccataatctaactacaattacgaaacctctaaaatactcatatataaataaatgctctcggttgttgtcagacgatcgaaccgaggtgccccagctggttaatgccaatcaatactctccttgcgtatcgatagtgccgtctacggtttgggaagacggtgattactaccggaagcaactgtccccccttgaaggtggtggttggcttgttgcatacgggtcaacggtagccatgacggagcagctccagatgggctttggaataacagtacagtatgggaccgacacgaactctgtatgcccaaagctatcacgcgccctggttccaaggggctcttcagctcatcatcaccatcatcatcatcaccatcactgaggatcccctcgccccggacctgccctcccgccaggtgcacccacctgcaataaatgcagcgaagccgggaaatatt

SEQ ID NO: 36 - DNA, 1703 bp, Artificial Sequence
  C19DP-MR-#8
agatcttaatacgactcactatagggaaataagacgcgcctagcagtgtcccagccgggttcgtgtcgccgaattcgccaccatgggtgtgaaagtcctatttgcactaatttgtattgccgtggctgaagcaggggcggcgccgactgagtccatcgtgcggtttcctaacataactaacctctgtccatttggggaagtatttaatgcaacccggtttgcatcggtgtacgcgtggaatcgcaaaagaatatccaactgtgttgccgattactcagttctgtacaactcagcttcattctcaactttcaaatgttacggggtttcacctaccaagctcaatgacctctgttttactaacgtctatgcagactcatttgtgatccgcggagatgaagtccgccaaattgctcccggccaaactggcaacatagcggattacaattataagctcccagatgattttacaggatgcgtcattgcatggaattccaataatctcgactctaaggtgggtggaaattacaattatcgttaccggctattccggaaatcaaatctgaaaccttttgaacgtgatatatcaacagagatctaccaagccggaagtaagccttgcaacggggtggagggcttcaactgctactttcctcttcagtcgtatggatttcaacccactaacggagttggctatcaaccatatcgcgtagtagtcctctcattcgaactactacacgcacccgcaacggtgacatcagcggaggcggccgcgaaagaggctgcagctaaagaagcagccgctaaggaagctgctgccaaggcccttgaagcagaggctgctgcgaaggaagcggccgcgaaggaagcggccgccaaggaagcagccgctaaggcagaagccaagccatcaggatccgtagtggaacaagcagagggtgtggaatgcgatttctctccgcttctgtcaggcactccaccccaggtttataattttaagcgactagtattcaccaattgtaattacaacctaaccaaactactgtcgctattttctgtaaacgatttcacctgctcccagatctcaccggcagctatagcttcgaattgctactcatcactgatcctagattacttcagctatccgttgtctatgaaatccgacctgtcagtttcttctgccggtccaatctctcaattcaattacaaacaatctttctctaaccccacttgcctaattctggccacggtcccacataatcttacaaccattactaagcctcttaaatattcttatattaacaaatgctctcggttgttgtcagacgaccggactgaggtaccccaacttgttaacgccaaccagtactcgccatgcgtctccatcgtaccgtcaacagtgtgggaagacggagattactatcggaaacagctctcgccacttgaaggcggcggatggctggtagcatccggatcaacagtagccatgacggagcagctccagatgggattcggaatcactgtgcagtatggaaccgacactaattcagtgtgccccaaactatctcgagccctggttccaaggggctcttcagctcatcatcaccatcatcatcatcaccatcactgaggatcccctcgccccggacctgccctcccgccaggtgcacccacctgcaataaatgcagcgaagccgggaaatatt

SEQ ID NO: 37 - DNA, 1703 bp, Artificial Sequence
  C19DP-MR-#9
agatcttaatacgactcactatagggaaataagacgcgcctagcagtgtcccagccgggttcgtgtcgccgaattcgccaccatgggggttaaagtgctttttgctctaatttgcatcgcagtggcggaagcaggtgcagcaccaacagagtcaatagtccgatttccaaacataacaaacctttgcccctttggtgaggtattcaacgctactcgatttgcatctgtatacgcttggaaccgcaaaagaatatccaactgtgtcgcggactattcagttctatacaactctgcgtccttttcaaccttcaagtgctatggtgtgtcccctacgaaactcaatgacctttgttttaccaatgtctacgcggactcatttgtcatacgcggagatgaagtacggcaaatcgctcctggacaaactggcaacatagcggattataactataaacttcctgacgactttaccgggtgcgtaattgcatggaactctaacaaccttgactctaaagtgggcggcaactataattaccgctaccgtctattccgaaagtccaatcttaaacccttcgaacgagacatatccaccgagatataccaagccggaagtaagccttgcaacggggttgaaggctttaactgttacttccctctccaatcatatggcttccaacctacgaacggtgtaggttatcagccatatcgagtagtagttctttcctttgaactgctgcatgctccggcaacagtcacatccgcggaggcagcggcaaaagaggctgcagctaaagaagccgcagcaaaagaggcagccgcaaaagcactggaagcagaggccgctgcgaaggaggcggcagcaaaagaagcagctgcaaaggaggctgctgctaaagcggaagccaagccttcgggctctgtcgtcgaacaagcagaaggtgtagagtgtgacttctctccgcttctgtcaggcacccccccacaggtctataactttaagcgactggtttttacaaattgtaattacaaccttactaagctactatcgctattctcggtcaacgatttcacgtgttctcaaatctctcccgccgccattgcgtccaactgttattcatcccttatactcgattacttcagctatccgttgtccatgaaatcagacctgtcggtatcctcagctggacctatctcacagttcaactataaacagtccttttcgaaccccacatgtcttatacttgctaccgtccctcacaatcttaccactataactaaaccactgaaatattcttatatcaataagtgctctcggttgttgtcagacgaccgaacggaggtaccacaactcgtcaacgccaatcaatattcaccatgtgtatccatcgtcccatcaacagtgtgggaggatggtgattattatcgtaagcaactgtcaccgcttgaaggaggaggttggctggtagcgtctgggtccaccgtagccatgacggagcagctccagatgggatttggaataaccgtccaatacgggactgataccaattcagtttgccccaaactctcccgcgccctggttccaaggggctcttcagctcatcatcaccatcatcatcatcaccatcactgaggatcccctcgccccggacctgccctcccgccaggtgcacccacctgcaataaatgcagcgaagccgggaaatatt

SEQ ID NO: 38 - DNA, 1703 bp, Artificial Sequence
  C19DP-MR-#17
agatcttaatacgactcactatagggaaataagacgcgcctagcagtgtcccagccgggttcgtgtcgccgaattcgccaccatgggcgtcaaagtactattcgctcttatctgtatagccgtagcagaggcaggagccgcaccaacagaatctatcgtgcgatttccaaatataactaatctttgcccctttggtgaggtatttaacgcgacacgattcgcttccgtatacgcctggaaccgcaaaagaatatccaactgtgtggcggattactccgtcctctacaattctgcctccttctctacgtttaaatgttatggagtgtcaccgacaaaacttaatgacctgtgctttacaaacttttatgcagactcattcgttatacggggtgacgaggtacgacaaattgcgcctggccaaactggcaacatagcggattataactacaaactacctgacgatttcacggggtgcgtcatcgcctggaattcaaataacctggactcaaaagtcggaggtaactacaactaccgctatcgtctattccgaaagtcaaatctgaaaccctttgagcgcgacatttctaccgagatctaccaagccggaagtaagccttgtaatggcgttgagggctttaattgctattttccactccaatcatacggattccaacctacaaatggtgtaggttatcaaccatatcgagttgtagttctttcatttgagcttcttcatgcccccgcgacagttacatcagccgaagccgctgccaaagaggctgcagctaaagaagccgccgctaaagaagcagctgcaaaggctctcgaagcggaagctgccgccaaagaagcagctgcaaaggaagcagctgctaaagaagcggcagcgaaggccgaggcaaaaccatccggttccgttgtggaacaggcagaaggggtagagtgcgacttctctccgcttctgtcaggcaccccaccccaagtctacaacttcaagcgtcttgtattcaccaattgcaactataatctaaccaaacttctttccctcttctctgtaaatgatttcacgtgttcacaaatctctccggcagccatcgcctcgaattgctattcctctcttatcctggattacttcagctatccgttgtccatgaaatccgacctctctgtttcttctgcaggccctatatcccaatttaattataagcagtccttttcaaacccaacttgtctaattcttgccacagtacctcacaatctaactactattacaaagccactaaaatactcgtatattaataagtgctctcggttgttgtcagacgaccgtacagaggtacctcaactagtgaacgccaaccagtactcaccatgtgtatcgatagtaccgtccacagtctgggaggatggagattactatcggaaacagctgtcacctctagagggaggaggatggcttgtggcgtcaggctcaaccgttgccatgacggagcagctccagatgggcttcggtatcactgtgcagtatggaaccgatacaaactcagtatgtccaaaactatcccgagccctggttccaaggggctcttcagctcatcatcaccatcatcatcatcaccatcactgaggatcccctcgccccggacctgccctcccgccaggtgcacccacctgcaataaatgcagcgaagccgggaaatatt

SEQ ID NO: 39 - DNA, 1703 bp, Artificial Sequence
  C19DP-MR-#29
agatcttaatacgactcactatagggaaataagacgcgcctagcagtgtcccagccgggttcgtgtcgccgaattcgccaccatgggtgtaaaagttctgtttgccctaatctgcatagcggtagccgaagctggtgccgcaccaacagagtcaatagttcgttttccgaacattacaaacctgtgtcccttcggcgaggtattcaatgcaacacgatttgcatccgtctacgcctggaaccgcaaaagaatatccaactgtgttgcagattactctgtcctctataattccgcatccttttcaacattcaaatgctacggggtgtcccctactaaactaaacgacctatgttttacgaacgtatatgccgactcatttgtgattcgcggagatgaggtgcgccagattgcccccgggcaaactggcaacatagcggattacaattacaaacttcccgatgacttcacgggttgcgtcatcgcatggaactcgaataacctggactccaaagtcggagggaattacaattaccgttatcgactttttcgtaaatctaacctcaagccctttgaacgtgacatatcaacggaaatataccaagccggaagtaagccttgcaatggggtagaaggattcaattgctatttcccccttcagtcttacggttttcagcctacaaatggagtaggatatcaaccctaccgagtggtcgtactatcgtttgagctacttcacgcgcccgccactgttacttctgctgaagctgctgcaaaagaggctgcagctaaagaagcagctgcgaaggaagccgcggctaaggctctcgaagcagaggccgccgtgaaagaagctgcagctaaagaagcagcagcaaaagaagctgctgctaaggcagaggctaaaccctcgggatcagtggtagaacaagccgaaggagtggagtgcgacttctctccgcttctgtcaggcactccaccacaagtctacaattttaagcgactcgtcttcacaaattgtaactataaccttacgaaactcctatcactgttttcggtaaatgactttacttgttcccagatctcccccgccgcaatcgcatcaaattgttactcttctctaatactggattacttcagctatccgttgtcgatgaagtccgatctatccgtttcgtcagctggcccgatatcgcaatttaactacaaacaatctttctctaaccctacatgtctaattctagccactgttccacacaacctaacgacaattacgaaaccactcaaatattcatatattaacaaatgctctcggttgttgtcagacgaccgaacggaggtaccccagctcgttaacgccaaccagtattctccgtgtgtatcaatagtcccatccaccgtgtgggaagatggggattactaccgcaagcagctgtcgcccctggagggcggaggatggctggtagcatcaggttcaaccgttgccatgacggagcagctccagatggggtttgggataactgtgcagtatggaactgacacaaactccgtttgtcctaaactgtctcgagccctggttccaaggggctcttcagctcatcatcaccatcatcatcatcaccatcactgaggatcccctcgccccggacctgccctcccgccaggtgcacccacctgcaataaatgcagcgaagccgggaaatatt

SEQ ID NO: 40 - DNA, 1703 bp, Artificial Sequence
  C19DP-MR-#41
agatcttaatacgactcactatagggaaataagacgcgcctagcagtgtcccagccgggttcgtgtcgccgaattcgccaccatgggggttaaagtactgtttgcgctgatctgtatcgctgtagccgaggcgggagcggcaccgacagagtcaatagtccgatttcccaatataacgaatctatgtccgttcggtgaagtatttaatgccacacgctttgcttcagtatatgcatggaaccgcaaaagaatatccaactgtgtggcagactactccgtactctacaactcagcgtcattctcaacatttaaatgctatggggtctcacctaccaagctaaacgatctatgttttacgaacgtatatgcagattcattcgtaatacgtggtgacgaagtacgacaaatagcaccgggccaaactggcaacatagcggattacaactataaactgccagatgactttaccgggtgcgttatcgcatggaattcgaataacctggactccaaggtaggtggaaattataactatcgttaccgactctttcggaagtcaaatcttaaaccatttgaacgagatatttcaactgaaatttaccaagccggaagtaagccttgtaatggagtagaagggttcaactgttactttcccctccaatcctatggcttccagccgacaaatggtgttggatatcaaccatatcgagtcgttgtactgtctttcgaactgctacatgcccctgcgactgtcacctctgcggaggcagccgctaaagaggctgcagctaaagaagccgcggctaaagaggcagcggccaaggcacttgaggcggaggcagctgcaaaggaagccgcagccaaagaagcagcagcaaaggaagcagcagccaaagcagaagcgaaaccctcagggtcggtagtcgaacaagccgaaggagttgaatgtgacttctctccgcttctgtcaggcacgccaccccaagtctataacttcaaacgacttgtttttacaaattgtaattataatctcacaaaactactgtcactattttcagttaacgatttcacttgttcgcaaatctccccggcagccatcgcgtcgaattgctactcatcgctgatcctcgattacttcagctatccgttgtctatgaagtctgacctgtcagtttcgtccgccggtccaatatctcaatttaattataaacaatcgttttcaaatccaacatgtctgatccttgccacagtaccacacaaccttacaacgatcacaaaaccgctaaaatattcatatattaataaatgctctcggttgttgtcagacgaccgcacagaagtgccacaattagtaaacgctaaccagtattccccgtgtgtgtcgatagtaccatcaacggtctgggaggacggtgactattatcgtaaacagctatcgcctctggagggaggggggtggctagtagcgtcaggttcaacggtagccatgacggagcagctccagatgggctttggtatcaccgtccaatacggaacagacacaaattccgtatgtcccaaactgtcacgggccctggttccaaggggctcttcagctcatcatcaccatcatcatcatcaccatcactgaggatcccctcgccccggacctgccctcccgccaggtgcacccacctgcaataaatgcagcgaagccgggaaatatt